European Patent Specification EP 2 774 615 B1, published February 12, 2025. Title: MUSCLE VOLUME INCREASING AGENT. Applicant: KAO CORPORATION. The sequence listing filed with the application follows.

SEQUENCE LISTING (12 sequences)

SEQ ID NO: 1 - DNA, 20 bp, Artificial Sequence
  Primer sequence specific to IGF-1
agttcgtgtgtggaccgagg

SEQ ID NO: 2 - DNA, 20 bp, Artificial Sequence
  Primer sequence specific to IGF-1
cagctccggaagcaacactc

SEQ ID NO: 3 - DNA, 21 bp, Artificial Sequence
  Primer sequence specific to Atrogin-1
gcagcagctgaatagcatcca

SEQ ID NO: 4 - DNA, 21 bp, Artificial Sequence
  Primer sequence specific to Atrogin-1
ggtgatcgtgaggcctttgaa

SEQ ID NO: 5 - DNA, 21 bp, Artificial Sequence
  Primer sequence specific to MuRF1
aatgtagaagcctccaagggc

SEQ ID NO: 6 - DNA, 20 bp, Artificial Sequence
  Primer sequence specific to MuRF1
ctgtcccaaagtcaatggcc

SEQ ID NO: 7 - DNA, 19 bp, Artificial Sequence
  Primer sequence specific to Myh1
gctagtaacatggaggtca

SEQ ID NO: 8 - DNA, 22 bp, Artificial Sequence
  Primer sequence specific to Myh1
taaggcactcttggcctttatc

SEQ ID NO: 9 - DNA, 21 bp, Artificial Sequence
  Primer sequence specific to Dok-7
tgagcttcctgtttgactgca

SEQ ID NO: 10 - DNA, 20 bp, Artificial Sequence
  Primer sequence specific to Dok-7
gcaacacgctcttctgaggc

SEQ ID NO: 11 - DNA, 21 bp, Artificial Sequence
  Primer sequence specific to MuSK
catggcagagtttgacaaccc

SEQ ID NO: 12 - DNA, 22 bp, Artificial Sequence
  Primer sequence specific to MuSK
ttcggaggaactcattgaggtc